European Patent Specification EP 4 001 438 B1, published May 15, 2024. Title: COMPOSITION FOR DETECTING LEPTOSPIROSIS AND METHOD OF DIAGNOSING. Applicant: Industry Academic Cooperation Foundation of Chosun University. The sequence listing filed with the application follows.

SEQUENCE LISTING (27 sequences)

SEQ ID NO: 1 - DNA, 18 bp, Artificial Sequence
  IS1500-290F primer
gattgccacaacagattc

SEQ ID NO: 2 - DNA, 18 bp, Artificial Sequence
  IS1500-475R primer
aatcgaccaacccactac

SEQ ID NO: 3 - DNA, 23 bp, Artificial Sequence
  IS1500-anti-312P probe
agttcggagcaacccgattccca

SEQ ID NO: 4 - DNA, 18 bp, Artificial Sequence
  IS1500-QF primer
cttgctccgtaaattgaa

SEQ ID NO: 5 - DNA, 18 bp, Artificial Sequence
  IS1500-QR primer
gtctcgttcaggattcta

SEQ ID NO: 6 - DNA, 21 bp, Artificial Sequence
  IS1500-QP probe
ccgaagcaaccgaactaagcc

SEQ ID NO: 7 - DNA, 18 bp, Artificial Sequence
  lepto-IS1500_567F primer
caaggaaaacaggagaaa

SEQ ID NO: 8 - DNA, 18 bp, Artificial Sequence
  lepto-IS1500_719R primer
cccgaaagagratcttaa

SEQ ID NO: 9 - DNA, 24 bp, Artificial Sequence
  lepto-IS1500_590P probe
tcggattgccacaacagattctaa

SEQ ID NO: 10 - DNA, 18 bp, Artificial Sequence
  lepto-IS1500_567F primer
caaggaaaacaggagaaa

SEQ ID NO: 11 - DNA, 20 bp, Artificial Sequence
  lepto-IS1500_747R primer
gatccagtattacacaaaga

SEQ ID NO: 12 - DNA, 24 bp, Artificial Sequence
  lepto-IS1500_590P probe
tcggattgccacaacagattctaa

SEQ ID NO: 13 - DNA, 18 bp, Artificial Sequence
  lepto-IS1500_567F primer
caaggaaaacaggagaaa

SEQ ID NO: 14 - DNA, 18 bp, Artificial Sequence
  lepto-IS1500_758R primer
tcgagaataaagatccag

SEQ ID NO: 15 - DNA, 24 bp, Artificial Sequence
  lepto-IS1500_590P probe
tcggattgccacaacagattctaa

SEQ ID NO: 16 - DNA, 18 bp, Artificial Sequence
  IS1500-55F primer
gtgtctcgttcaggattc

SEQ ID NO: 17 - DNA, 19 bp, Artificial Sequence
  IS1500-230R primer
gttcttgctccgtaaattg

SEQ ID NO: 18 - DNA, 21 bp, Artificial Sequence
  IS1500-anti-192P probe
ccgaagcaaccgaactaagcc

SEQ ID NO: 19 - DNA, 20 bp, Artificial Sequence
  IS1500-459F primer
agtgggttggtcgatttcaa

SEQ ID NO: 20 - DNA, 21 bp, Artificial Sequence
  IS1500-557R primer
tggatcctcgatccgaatgaa

SEQ ID NO: 21 - DNA, 23 bp, Artificial Sequence
  IS1500-500P probe
tgtgcaccgctctttccaaagca

SEQ ID NO: 22 - DNA, 843 bp, Artificial Sequence
  L. interrogans IS 1500 gene sequence
atggaaactcatcgatttgagtattcgattcaaagcatggctaacgttttaggagtgtctcgttcaggattctatcaatttctaaaacggagtaaaaacgaattagaaaaatataatcctgaacttgtcgagttcattcgggaaacgtggctaacaagccgtaagaattacggcttagttcggttgcttcgggaagtgaagaaagtgtattcaatttacggagcaagaacggttcgaaaagtgatgaaactttgtgaaattcaaggaaaacaggagaaacgttttcggattgccacaacagattctaatcatgggaatcgggttgctccgaacttagttcaacggaatttcaaaccgaatcagaagaatcggatctgggtttcagatattacttttttaagatcctctttcgggtggatttatctttgtgtaatactggatctttattctcgaaaagtagtgggttggtcgatttcaaattctaatgattctaagttagtgtgcaccgctctttccaaagcaatcgaatgtagaaatcctcctaagggtttagtttttcattcggatcgaggatccaattattgttcgtacgaaactcgaaggtatctgttaaataataaactaagaaggagtaatagtagaaagggaaattgttgggacaacgcagtcgctgagtccttctttggttctctgaaaagagaaatggaatataattacttttataaaattcaagaagccgaagaattactttttgatcatatagaggtttattataatagacacagatctcattcgtcattagactttgtgagtcctgtgcaatttgaagtaaatgctgcgtaa

SEQ ID NO: 23 - DNA, 187 bp, Artificial Sequence
  PCR product
gattgccacaacagattctaatcatgggaatcgggttgctccgaacttagttcaacggaatttcaaaccgaatcagaagaatcggatctgggtttcagatattacttttttaagatcctctttcgggtggatttatctttgtgtaatactggatctttattctcgaaaagtagtgggttggtcgatt

SEQ ID NO: 24 - DNA, 21 bp, Artificial Sequence
  Adia 217F primer
ccgtgattttcctaactaagg

SEQ ID NO: 25 - DNA, 22 bp, Artificial Sequence
  Adia 218R primer
cagattacttagtcgcgtcaga

SEQ ID NO: 26 - DNA, 20 bp, Artificial Sequence
  Lepto A primer
ggcggcgcgtcttaaacatg

SEQ ID NO: 27 - DNA, 21 bp, Artificial Sequence
  Lepto B primer
ttccccccattgagcaagatt